European Patent Specification EP 3 524 063 B1, published April 26, 2023. Title: METHOD OF MANUFACTURING SEASONING AGENT CONTAINING NUCLEIC ACIDS. Applicant: AMANO ENZYME INC. The sequence listing filed with the application follows.

SEQUENCE LISTING (19 sequences)

SEQ ID NO: 1 - protein, 424 aa, Penicillium multicolor
MAPKKIIIDTDPGIDDILALLLALSSKPEDVEILLISLTFGNIEVKNCLRNVVSMFHILEREIQWRRGNGKSEGYGTMRAFRPVVAVGAEDPLEDQKMLADYFHGTDGLGGIHASHPHLTPSKAWEHLFTPAVDPQGIEPVQTGAGPGDHSFIPSRLPAHKEILRALRQNEPDTVTLVAVGPLTNLALAAAEDPETFLRVKEVVVMGGAINQPGNVTPVGEFNAYADAVAAARVFALTSPNPNSTLPPTTSPLLGLYPAKLSRQLTLRLFPLDITLRHNLSRGQFRQAVEPLLATGSPLAEWVTAFMGHTFRTLERLHPGHEGDEAQLSLHDPVCVWYALTAEDSHWTPSANSPEDIRVETLGQWTRGMCVIDGRNRHKIDGDEESSSDHGLWLSARAGNRILRMDGSPAEHTFGKILIDRIFH

SEQ ID NO: 2 - protein, 380 aa, Penicillium multicolor
MHFPVSLPLLCGSLLPLITGTLAVPKASRADKHYAIMDNDWYTAGFVPYLIALDGDVEVLGLASDTANTWQPQVALHAVATLEAGNLSCIPVYPGSTWPLINTPNRFQAWEMVHGKLPWEGAFAPENKTLEAEGNDPTSGNPNRIVKAAFKEGFPKGKPENRTSAANFMVEMVHKYPGQVSIYSAGALTNVALAVRMDPQFASLAKELVIMGGYVDLNMLQATGSVLLADLQSDINLMIDPEASKIALTAEFPNITIAGNVANQVFPTKEFVDEIASVPNPYSKLFHDYYDLSFPFWDETAAALMVDPTLATNQTSVFLDVDTAYGSPNYGNIHVYQKALAPVGIREVNFVFQVDGDRLKQRIKHSLQYPKSCADLRNER

SEQ ID NO: 3 - DNA, 1275 bp, Penicillium multicolor
atggcacctaagaaaatcatcattgacactgacccgggtatcgatgacatcctggcactgctgctggctctgtcatctaagccagaggatgttgagattctacttatctctttaacatttggaaacattgaggtgaagaactgtcttcgaaatgtggtctccatgtttcatatcctcgagcgcgagatccagtggcgtcgtggtaacggcaagtccgaaggctatggcactatgcgtgctttccgcccagtagtagccgtgggagcggaagatcccttggaagaccagaagatgctcgctgattatttccatggaaccgatggccttggtggcatccatgctagtcacccacatctcactccaagcaaggcctgggagcatctattcaccccggccgtggatccccaggggatcgagcctgtgcaaacgggagctggtcccggcgaccattcctttatcccatcaagactacctgcacacaaggagattcttcgtgcactgcgccagaatgagcctgacaccgtgactctcgtggcggttggtccactgaccaacttggccttggcagcagcagaggatcccgaaaccttcctacgtgtcaaggaggtcgttgtgatgggtggagcaatcaaccagcctggaaatgtcacccccgttggagaattcaacgcctacgcagacgccgttgcagctgcgcgagtctttgcgctgacatcacctaatcccaactcgactctaccaccgaccacgagtccactacttggcctgtaccctgcaaagctcagccgacaattgactctgcgtctcttcccgctggacatcaccctgcgccataacctgtcccgcggccaattccgccaagcagttgagcctctcctcgcaacaggctcacccctcgctgaatgggtgacagcattcatgggacacacgttccgaaccctggaacgcctgcaccccggccatgagggcgatgaagcccagctgagtctccacgaccctgtctgtgtgtggtatgcccttacagcagaggattcgcactggactccctccgccaattccccagaggacattcgtgttgagacattgggccagtggacgcgtggtatgtgcgtaatcgatggccgaaaccgccataagattgatggcgacgaggaaagctcgagtgatcatggtctgtggttgagtgctcgtgcaggaaaccgcattttgcgaatggatggatcgccagccgaacacacgttcggcaagatcctcatcgatagaatcttccactaa

SEQ ID NO: 4 - DNA, 1016 bp, Penicillium multicolor
gtacccattttctaacactatctggacagcacccacatctcactccaagcaaggcctgggagcatctattcaccccggccgtggatccccaggggatcgagcctgtgcaaacgggagctggtcccggcgaccattcctttatcccatcaagactacctgcacacaaggagattcttcgtgcactgcgccagaatgagcctgacaccgtgactctcgtggcggttggtccactgaccaacttggccttggcagcagcagaggatcccgaaaccttcctacgtgtcaaggaggtcgttgtgatgggtggagcaatcaaccagcctggaaatgtatgaaccccgtcgaaacacccatttgataataagtcattaaccgcgattgactaggtcacccccgttggagaattcaacgcctacgcagacgccgttgcagctgcgcgagtctttgcgctgacatcacctaatcccaactcgactctaccaccgaccacgagtccactacttggcctgtaccctgcaaagctcagccgacaattgactctgcgtctcttcccgctggacatcaccctgcgccataacctgtcccgcggccaattccgccaagcagttgagcctctcctcgcaacaggctcacccctcgctgaatgggtgacagcattcatgggacacacgttccgaaccctggaacgcctgcaccccggccatgagggcgatgaagcccagctgagtctccacgaccctgtctgtgtgtggtatgcccttacagcagaggattcgcactggactccctccgccaattccccagaggacattcgtgttgagacattgggccagtggacgcgtggtatgtgcgtaatcgatggccgaaaccgccataagattgatggcgacgaggaaagctcgagtgatcatggtctgtggttgagtgctcgtgcaggaaaccgcattttgcgaatggatggatcgccagccgaacacacgttcggcaagatcctcatcgatagaatcttccactaa

SEQ ID NO: 5 - DNA, 1143 bp, Penicillium multicolor
atgcatttccctgtttcattgccgctgttgtgcggctctttgctgcctctcatcaccggcaccctggcagtgcccaaggcctcgcgtgccgacaagcactatgccatcatggacaatgattggtacacagcgggtttcgtgccttacctgatcgccctcgatggcgatgtggaggttctgggcctagcctctgacaccgcaaacacctggcagcctcaggtcgctctgcacgctgtcgcaactctggaagctggcaacttgagctgtatccccgtttacccaggctcgacatggccgctcatcaacacccccaaccgcttccaggcgtgggaaatggttcatggcaagctgccatgggagggtgcttttgcgccggagaacaagactctcgaggccgagggtaacgatcctacctctggcaaccccaaccgtatcgtcaaggccgctttcaaggaagggttccccaagggcaagcccgagaacagaacatctgctgccaacttcatggtcgagatggtgcacaagtaccccggccaggtctcgatctactctgctggagccctgaccaatgttgcgctggctgtgcgcatggatccccagtttgcatctctggctaaggagttggttatcatgggtggatacgtcgatttgaatatgctccaggccactggaagtgtcttgctggctgatcttcaatctgatatcaacttgatgattgatcccgaggcctccaagatcgcattgactgccgaattccccaatatcaccatcgccggtaacgtcgccaaccaggtctttcctaccaaggagttcgtcgacgagatcgcctccgttccaaacccctacagcaagctcttccacgactactacgatctgtccttccccttctgggatgagacggctgccgcgctgatggttgaccctactcttgctaccaaccagacctctgtcttcctcgacgtggataccgcttatggtagccccaactatggtaacattcacgtttaccagaaggctcttgcccctgttggtatccgggaggtcaactttgtcttccaggttgatggggatagacttaagcagcgcatcaagcactctctgcagtaccccaagtcatgcgccgacctgagaaatgagcgttga

SEQ ID NO: 6 - DNA, 847 bp, Penicillium multicolor
acgatcctacctctggcaaccccaaccgtatcgtcaaggccgctttcaaggaagggttccccaagggcaagcccgagaacagaacatctgctgccaacttcatggtcgagatggtgcacaagtaccccggccaggtctcgatctactctgctggagccctgaccaatgttgcgctggctgtgcgcatggatccccagtttgcatctctggctaaggagttggttatcatgggtggatacgtcgatttgaatatgctccaggccactggaagtgtcttgctggctgatcttcaatctgatgtatgtttcattcccggcttctatcagctgtgttcatctgctaacttctctttagatcaacttgatgattgatcccgaggcctccaagatcgcattgactgccgaattccccaatatcaccatcgccggtaacgtcgccaaccaggtctttcctaccaaggagttcgtcgacgagatcgcctccgttccaaacccctacagcaagctcttccacgactactacgatctgtccttccccttctgggatgagacggctgccgcgctgatggttgaccctactcttgctaccaaccagacctctggtgagtttaatctcgcattgacacttgtatgaacaaatctaacagcttatagtcttcctcgacgtggataccgcttatggtagccccaactatggtaacattcacgtttaccagaacgctcttgcccctgttggtatccgggaggtcaactttgtcttccaggttgatggggatagacttaagcagcgcatcaagcactctctgcagtaccccaagtcatgcgccgacctgagaaatgagcgttga

SEQ ID NO: 7 - protein, 15 aa, Penicillium multicolor
ADKHYAIMDNDWYTA

SEQ ID NO: 8 - protein, 15 aa, Penicillium multicolor
ADKHYAIMDNDWYTA

SEQ ID NO: 9 - protein, 9 aa, Penicillium multicolor
VETKLIFLT

SEQ ID NO: 10 - DNA, 20 bp, Artificial Sequence
  primer
  misc_feature (3)..(3): inosine
  misc_feature (6)..(6): g or a
  misc_feature (9)..(9): t or c
  misc_feature (10)..(10): a or c
  misc_feature (12)..(12): any of a, g, c, or t
  misc_feature (15)..(15): t or c
  misc_feature (16)..(16): t or c
  misc_feature (18)..(18): inosine
acnaartaymgnttyytnac

SEQ ID NO: 11 - DNA, 21 bp, Artificial Sequence
  primer
  misc_feature (4)..(4): any of a, g, c, or t
  misc_feature (7)..(7): any of a, g, c, or t
  misc_feature (9)..(9): g or t
  misc_feature (10)..(10): any of a, g, c, or t
  misc_feature (16)..(16): t or c
  misc_feature (19)..(19): any of a, g, c, or t
catnccnckngtccaytgncc

SEQ ID NO: 12 - DNA, 26 bp, Artificial Sequence
  primer
  misc_feature (3)..(3): any of a, g, c, or t
  misc_feature (6)..(6): a, c, or t
  misc_feature (12)..(12): t or c
  misc_feature (15)..(15): t or c
  misc_feature (18)..(18): t or c
  misc_feature (24)..(24): t or c
gcnathatggayaaygaytggtayac

SEQ ID NO: 13 - DNA, 23 bp, Artificial Sequence
  primer
  misc_feature (3)..(3): any of a, g, c, or t
  misc_feature (6)..(6): any of a, g, c, or t
  misc_feature (9)..(9): t or c
  misc_feature (12)..(12): g or a
  misc_feature (18)..(18): g or a
  misc_feature (21)..(21): any of a, g, c, or t
gcngcngtytcrtcccaraangg

SEQ ID NO: 14 - DNA, 25 bp, Artificial Sequence
  primer
atggcacctaagaaaatcatcattg

SEQ ID NO: 15 - DNA, 25 bp, Artificial Sequence
  primer
ttagtggaagattctatcgatgagg

SEQ ID NO: 16 - DNA, 25 bp, Artificial Sequence
  primer
atgcatttccctgtttcattgccgc

SEQ ID NO: 17 - DNA, 23 bp, Artificial Sequence
  primer
tcaacgctcatttctcaggtcgg

SEQ ID NO: 18 - DNA, 574 bp, Artificial Sequence
  probe
gaggatcccgaaaccttcctacgtgtcaaggaggtcgttgtgatgggtggagcaatcaaccagcctggaaatgtatgaaccccgtcgaaacacccatttgataataagtcattaaccgcgattgactaggtcacccccgttggagaattcaacgcctacgcagacgccgttgcagctgcgcgagtctttgcgctgacatcacctaatcccaactcgactctaccaccgaccacgagtccactacttggcctgtaccctgcaaagctcagccgacaattgactctgcgtctcttcccgctggacatcaccctgcgccataacctgtcccgcggccaattccgccaagcagttgagcctctcctcgcaacaggctcacccctcgctgaatgggtgacagcattcatgggacacacgttccgaaccctggaacgcctgcaccccggccatgagggcgatgaagcccagctgagtctccacgaccctgtctgtgtgtggtatgcccttacagcagaggattcgcactggactccctccgccaattccccagaggacattcgtgttgagacattgggcc

SEQ ID NO: 19 - DNA, 509 bp, Artificial Sequence
  probe
agacaccgcaaacacctggcagcctcaggtcgctctgcacgctgtcgcaactctggaagctggcaacttgagctgtatccccgtttacccaggctcgacatggccgctcatcaacacccccaaccgcttccaggcgtgggaaatggttcatggcaagctgccatgggagggtgcttttgcgccggagaacaagactctcgaggccgagggtaacgatcctacctctggcaaccccaaccgtatcgtcaaggccgctttcaaggaagggttccccaagggcaagcccgagaacagaacatctgctgccaacttcatggtcgagatggtgcacaagtaccccggccaggtctcgatctactctgctggagccctgaccaatgttgcgctggctgtgcgcatggatccccagtttgcatctctggctaaggagttggttatcatgggtggatacgtcgatttgaatatgctccaggccactggaagtgtcttgctggctgatcttcaatctg